European Patent Application EP 4 592 312 A1, published July 30, 2025. Title: NOVEL ANTIBODY FOR PREVENTION OR TREATMENT OF FIBROTIC DISEASE. Applicant: Industry-Academic Cooperation Foundation, Yonsei University. Application EP. The sequence listing filed with the application follows.

SEQUENCE LISTING (38 sequences)

SEQ ID NO: 1 - protein, 8 aa, synthetic construct
GFTFSDYW

SEQ ID NO: 2 - protein, 11 aa, synthetic construct
IRNKPYNYETY

SEQ ID NO: 3 - protein, 12 aa, synthetic construct
TAYYRYDVLFDY

SEQ ID NO: 4 - protein, 6 aa, synthetic construct
QDISNY

SEQ ID NO: 5 - skipped

SEQ ID NO: 6 - protein, 9 aa, synthetic construct
QQSKTLPLT

SEQ ID NO: 7 - protein, 25 aa, synthetic construct
EVKLVETGGGLVQPGRPMKLSCVAS

SEQ ID NO: 8 - protein, 17 aa, synthetic construct
MNWVRQSPEKGLEWVVQ

SEQ ID NO: 9 - protein, 38 aa, synthetic construct
YYSDSVKGRFTISRDDSKSCVYLQMNNLRAEDMGIYYC

SEQ ID NO: 10 - protein, 11 aa, synthetic construct
WGQGTSLTVSS

SEQ ID NO: 11 - protein, 121 aa, synthetic construct
EVKLVETGGGLVQPGRPMKLSCVASGFTFSDYWMNWVRQSPEKGLEWVVQIRNKPYNYETYYSDSVKGRFTISRDDSKSCVYLQMNNLRAEDMGIYYCTAYYRYDVLFDYWGQGTSLTVSS

SEQ ID NO: 12 - protein, 26 aa, synthetic construct
DIQMTQTTSSLSASLGDRVTISCRAS

SEQ ID NO: 13 - protein, 17 aa, synthetic construct
LNWYQQKPEGTVKLLIY

SEQ ID NO: 14 - protein, 36 aa, synthetic construct
RLHSGVPSRFSGSGSGTDYSLTISNLEQEDIATYFC

SEQ ID NO: 15 - protein, 10 aa, synthetic construct
FGAGTKLELK

SEQ ID NO: 16 - protein, 107 aa, synthetic construct
DIQMTQTTSSLSASLGDRVTISCRASQDISNYLNWYQQKPEGTVKLLIYYTSRLHSGVPSRFSGSGSGTDYSLTISNLEQEDIATYFCQQSKTLPLTFGAGTKLELK

SEQ ID NO: 17 - DNA, 24 bp, synthetic construct
  source 1..24: mol_type = other DNA
ggattcacttttagtgactactgg

SEQ ID NO: 18 - DNA, 30 bp, synthetic construct
  source 1..30: mol_type = other DNA
attagaaacaaaccttataattatgaaaca

SEQ ID NO: 19 - DNA, 36 bp, synthetic construct
  source 1..36: mol_type = other DNA
acagcctactataggtacgacgtcctcttcgactac

SEQ ID NO: 20 - DNA, 18 bp, synthetic construct
  source 1..18: mol_type = other DNA
caggacattagcaattat

SEQ ID NO: 21 - skipped

SEQ ID NO: 22 - DNA, 27 bp, synthetic construct
  source 1..27: mol_type = other DNA
caacagagtaaaacgcttcctctcacg

SEQ ID NO: 23 - DNA, 75 bp, synthetic construct
  source 1..75: mol_type = other DNA
gaggtgaagctggttgagactggaggaggcttggtgcaacctgggaggcccatgaaactctcctgtgttgcctct

SEQ ID NO: 24 - DNA, 51 bp, synthetic construct
  source 1..51: mol_type = other DNA
atgaactgggtccgccagtctccagagaaaggactggagtgggtagtacaa

SEQ ID NO: 25 - DNA, 114 bp, synthetic construct
  source 1..114: mol_type = other DNA
tattattcagattctgtgaaaggcagattcaccatctcaagagatgattccaaaagttgtgtctacctgcaaatgaacaacttaagagctgaagacatgggtatctattactgt

SEQ ID NO: 26 - DNA, 34 bp, synthetic construct
  source 1..34: mol_type = other DNA
tggggccaaggcacctctctcacagtctcctcag

SEQ ID NO: 27 - DNA, 364 bp, synthetic construct
  source 1..364: mol_type = other DNA
gaggtgaagctggttgagactggaggaggcttggtgcaacctgggaggcccatgaaactctcctgtgttgcctctggattcacttttagtgactactggatgaactgggtccgccagtctccagagaaaggactggagtgggtagtacaaattagaaacaaaccttataattatgaaacatattattcagattctgtgaaaggcagattcaccatctcaagagatgattccaaaagttgtgtctacctgcaaatgaacaacttaagagctgaagacatgggtatctattactgtacagcctactataggtacgacgtcctcttcgactactggggccaaggcacctctctcacagtctcctcag

SEQ ID NO: 28 - DNA, 78 bp, synthetic construct
  source 1..78: mol_type = other DNA
gatatccagatgacacagactacatcctccctgtctgcctctctgggagacagagtcaccatcagttgcagggcaagt

SEQ ID NO: 29 - DNA, 51 bp, synthetic construct
  source 1..51: mol_type = other DNA
ttaaactggtatcagcagaaaccagaaggaactgttaaactcctgatctac

SEQ ID NO: 30 - DNA, 108 bp, synthetic construct
  source 1..108: mol_type = other DNA
agattacactcaggagtcccatcaagattcagtggcagtgggtctggaacagattattctctcaccattagcaacctggaacaagaagatattgccacttacttttgt

SEQ ID NO: 31 - DNA, 31 bp, synthetic construct
  source 1..31: mol_type = other DNA
ttcggagctgggaccaagttggagctgaaac

SEQ ID NO: 32 - DNA, 322 bp, synthetic construct
  source 1..322: mol_type = other DNA
gatatccagatgacacagactacatcctccctgtctgcctctctgggagacagagtcaccatcagttgcagggcaagtcaggacattagcaattatttaaactggtatcagcagaaaccagaaggaactgttaaactcctgatctactacacatcaagattacactcaggagtcccatcaagattcagtggcagtgggtctggaacagattattctctcaccattagcaacctggaacaagaagatattgccacttacttttgtcaacagagtaaaacgcttcctctcacgttcggagctgggaccaagttggagctgaaac

SEQ ID NO: 33 - DNA, 16 bp, synthetic construct
  source 1..16: mol_type = other DNA
cctcaagggctccaac

SEQ ID NO: 34 - DNA, 26 bp, synthetic construct
  source 1..26: mol_type = other DNA
ggttttgtattcaatcactgtcttgc

SEQ ID NO: 35 - DNA, 22 bp, synthetic construct
  source 1..22: mol_type = other DNA
tggtctgcaaggaatgcctgga

SEQ ID NO: 36 - DNA, 22 bp, synthetic construct
  source 1..22: mol_type = other DNA
tctttccctgggacaccatcag

SEQ ID NO: 37 - DNA, 20 bp, synthetic construct
  source 1..20: mol_type = other DNA
ctggcatcgtgctggactct

SEQ ID NO: 38 - DNA, 19 bp, synthetic construct
  source 1..19: mol_type = other DNA
gatctcggccagccagatc